European Patent Specification EP 3 322 726 B1, published March 12, 2025. Title: Sortilin D region antibodies. Applicant: H. Lundbeck A/S. The sequence listing filed with the application follows.

SEQUENCE LISTING (188 sequences)

SEQ ID NO: 1 - protein, 16 aa, Artificial
  5E1 CDR1 Light Chain
KSSQSLLDSNGKTYLN

SEQ ID NO: 2 - protein, 7 aa, Artificial
  5E1 CDR2 Light Chain
LVSKLDS

SEQ ID NO: 3 - protein, 9 aa, Artificial
  5E1 CDR 3 Light Chain
CQGTHFPLT

SEQ ID NO: 4 - protein, 10 aa, Artificial
  5E1 CDR 1 Heavy Chain
GFIFSIYGMS

SEQ ID NO: 5 - protein, 17 aa, Artificial
  5E1 CDR 2 Heavy Chain
MISSGGIYTQYPDSVKG

SEQ ID NO: 6 - protein, 8 aa, Artificial
  5E1 CDR 3 Heavy Chain
HDDSWFAY

SEQ ID NO: 7 - protein, 113 aa, Artificial
  5E1 VL
DVVMTQTPLTLSVTIGQPASISCKSSQSLLDSNGKTYLNWLLQRPGQSPKRLIYLVSKLDSGVPDRFTGSGSGTDFTLRISRVEAEDLGVYYCCQGTHFPLTFGAGTKLELKR

SEQ ID NO: 8 - protein, 117 aa, Artificial
  5E1 VH
EVHLVESGGDLVNPGGSLKLSCEASGFIFSIYGMSWVRQTPDKRLEWVAMISSGGIYTQYPDSVKGRFTISRDNAKNTLYLQMSGLKSEDTGTYHCTRHDDSWFAYWGQGTLVTVSA

SEQ ID NO: 9 - protein, 14 aa, Artificial
  1F2 (Lambda) CDR1 Light Chain
RSSTGAVTTSNYAN

SEQ ID NO: 10 - protein, 7 aa, Artificial
  1F2 (Lambda) CDR2 Light Chain
GTNNRAP

SEQ ID NO: 11 - protein, 10 aa, Artificial
  1F2 (Lambda) CDR3 Light Chain
ALWYSNHFWV

SEQ ID NO: 12 - protein, 10 aa, Artificial
  1F2 (Lambda) CDR1 Heavy Chain
GFTFSSYGMS

SEQ ID NO: 13 - protein, 17 aa, Artificial
  1F2 (Lambda) CDR2 Heavy Chain
IISSGGSYTHYPDSVKG

SEQ ID NO: 14 - protein, 9 aa, Artificial
  1F2 (Lambda) CDR3 Heavy Chain
LCGPLCSGY

SEQ ID NO: 15 - protein, 112 aa, Artificial
  1F2 (Lambda) VL
QAVVTQESALTTSPGETVTLTCRSSTGAVTTSNYANWVQEKPDHLFTGLIGGTNNRAPGVPARFSGSLIGDKAALTITGAQTEDEAIYFCALWYSNHFWVFGGGTKLTVLGR

SEQ ID NO: 16 - protein, 118 aa, Artificial
  1F2 (Lambda) VH
EVQLVESGGDLVKPGGSLKLSCAASGFTFSSYGMSWVRQTPDKRLEWVAIISSGGSYTHYPDSVKGRFTISRDNAKNTLYLQMSSLKSEDTAMYYCARLCGPLCSGYWGQGTSVTVSS

SEQ ID NO: 17 - protein, 12 aa, Artificial
  068 CDR1 Light Chain
RASQSVSSNYLA

SEQ ID NO: 18 - protein, 7 aa, Artificial
  068 CDR2 Light Chain
GASSRAT

SEQ ID NO: 19 - protein, 9 aa, Artificial
  068 CDR3 Light Chain
QQYGSSPLT

SEQ ID NO: 20 - protein, 10 aa, Artificial
  068 CDR1 Heavy Chain
GFTFSIYGMH

SEQ ID NO: 21 - protein, 17 aa, Artificial
  068 CDR2 Heavy Chain
VISYDGSSKYYADSVKG

SEQ ID NO: 22 - protein, 11 aa, Artificial
  068 CDR3 Heavy Chain
DRALLTGVFDY

SEQ ID NO: 23 - protein, 108 aa, Artificial
  068 VL
EIVLTQSPGTLSLSPGERATLSCRASQSVSSNYLAWYQQKPGQAPRLLIYGASSRATGIPDRFSGSGSGTDFTLTISRLEPEDFAVYYCQQYGSSPLTFGGGTKVEIK

SEQ ID NO: 24 - protein, 120 aa, Artificial
  068 VH
QVQLVESGGGVVQPGRSLRLSCAASGFTFSIYGMHWVRQAPGKGLEWVAVISYDGSSKYYADSVKGRFTISRDNSKNTLYLQMNSLRAEDTAVYYCAKDRALLTGVFDYWGQGTLVTVSS

SEQ ID NO: 25 - protein, 11 aa, Artificial
  1320 CDR1 Light Chain
RASQSVSSYLA

SEQ ID NO: 26 - protein, 7 aa, Artificial
  1320 CDR2 Light Chain
DASNRAT

SEQ ID NO: 27 - protein, 9 aa, Artificial
  1320 CDR3 Light Chain
QQRTNWSIT

SEQ ID NO: 28 - protein, 10 aa, Artificial
  1320 CDR1 Heavy Chain
GFTFSSYVMS

SEQ ID NO: 29 - protein, 17 aa, Artificial
  1320 CDR2 Heavy Chain
AISGSGGSTYYADSVKG

SEQ ID NO: 30 - protein, 7 aa, Artificial
  1320 CDR3 Heavy Chain
LIWGWDI

SEQ ID NO: 31 - protein, 107 aa, Artificial
  1320 VL
EIVLTQSPATLSLSPGERATLSCRASQSVSSYLAWYQQRPGQAPRLLIYDASNRATGIPARFSGSGSGTDFTLSISSLEPEDFAVYYCQQRTNWSITFGQGTRLEIK

SEQ ID NO: 32 - protein, 116 aa, Artificial
  1320 VH
EVQLLESGGGLVQPGGSLRLSCAASGFTFSSYVMSWVRQAPGKGLEWVSAISGSGGSTYYADSVKGRFTISRDNSKNTLYLQMNSLRAEDTAVYYCAKLIWGWDIWGQGTMVTVSS

SEQ ID NO: 33 - protein, 12 aa, Artificial
  93-05 CDR1 Light Chain
RASQSVSSSYLA

SEQ ID NO: 34 - protein, 7 aa, Artificial
  93-05 CDR2 Light Chain
GASSRAT

SEQ ID NO: 35 - protein, 9 aa, Artificial
  93-05 CDR3 Light Chain
QQYGSSPFT

SEQ ID NO: 36 - protein, 10 aa, Artificial
  93-05 CDR1 Heavy Chain
GFTFSSYAMS

SEQ ID NO: 37 - protein, 17 aa, Artificial
  93-05 CDR2 Heavy Chain
AISGSGGSTYYADSVKG

SEQ ID NO: 38 - protein, 11 aa, Artificial
  93-05 CDR3 Heavy Chain
IAAAGTNYFDY

SEQ ID NO: 39 - protein, 108 aa, Artificial
  93-05 VL
EIVLTQSPGTLSLSPGERATLSCRASQSVSSSYLAWYQQKPGQAPRLLIYGASSRATGIPDRFSGSGSGTDFTLTISSLQPEDFAVYYCQQYGSSPFTFGPGTKVDIK

SEQ ID NO: 40 - protein, 120 aa, Artificial
  93-05 VH
VVQLLESGGGLVQPGGSLRLSCAASGFTFSSYAMSWVRQAPGKGLEWVSAISGSGGSTYYADSVKGRFTISRDNSMHTLFLQINSLRAEDTAVYYCVAIAAAGTNYFDYWGQGTLVTVSS

SEQ ID NO: 41 - protein, 12 aa, Artificial
  93-01 CDR1 Light Chain
RASQSVSSSYLA

SEQ ID NO: 42 - protein, 7 aa, Artificial
  93-01 CDR2 Light Chain
GASSRAT

SEQ ID NO: 43 - protein, 9 aa, Artificial
  93-01 CDR3 Light Chain
QQYGSSPFT

SEQ ID NO: 44 - protein, 10 aa, Artificial
  93-01 CDR1 Heavy Chain
GFTFSSYAMS

SEQ ID NO: 45 - protein, 17 aa, Artificial
  93-01 CDR2 Heavy Chain
AISGSGGSTYYADSVKG

SEQ ID NO: 46 - protein, 11 aa, Artificial
  93-01 CDR3 Heavy Chain
IAAAGTNYFDY

SEQ ID NO: 47 - protein, 108 aa, Artificial
  93-01 VL
EIVLTQSPGTLSLSPGERATLSCRASQSVSSSYLAWYQQKPGQAPRLLIYGASSRATGIPDRFSGSGSGTDFTLTISRLEPEDFAVYYCQQYGSSPFTFGPGTKVDIK

SEQ ID NO: 48 - protein, 120 aa, Artificial; identical to SEQ ID NO: 40
  93-01 VH

SEQ ID NO: 49 - protein, 12 aa, Artificial
  924 CDR1 Light Chain
RASQSVSSSYLA

SEQ ID NO: 50 - protein, 7 aa, Artificial
  924 CDR2 Light Chain
GASSRAT

SEQ ID NO: 51 - protein, 9 aa, Artificial
  924 CDR3 Light Chain
QQYGSSPIT

SEQ ID NO: 52 - protein, 12 aa, Artificial
  924 CDR1 Heavy Chain
GGSISSGNYYWN

SEQ ID NO: 53 - protein, 16 aa, Artificial
  924 CDR2 Heavy Chain
YIYYSGSTYYNPSLKS

SEQ ID NO: 54 - protein, 11 aa, Artificial
  924 CDR3 Heavy Chain
LITSQNFFFDY

SEQ ID NO: 55 - protein, 108 aa, Artificial
  924 VL
EIVLTQSPATLSLSPGERATLSCRASQSVSSSYLAWYQQKPGQAPRLLIYGASSRATGIPDRFSGSGSGTDFTLTISRLEPEDFAVYYCQQYGSSPITFGQGTRLEIK

SEQ ID NO: 56 - protein, 121 aa, Artificial
  924 VH
QVQLQESGPGLVKPSQTLSLTCTVSGGSISSGNYYWNWIRQHPGKGLEWIGYIYYSGSTYYNPSLKSRVTISVDTSKNQFSLKLNSVTSADTAVYYCAALITSQNFFFDYWGQGTLVTVSS

SEQ ID NO: 57 - protein, 12 aa, Artificial
  1276 CDR1 Light Chain
RASQSVSSSYLA

SEQ ID NO: 58 - protein, 7 aa, Artificial
  1276 CDR2 Light Chain
GASSRAT

SEQ ID NO: 59 - protein, 9 aa, Artificial
  1276 CDR3 Light Chain
QQYGSSPIT

SEQ ID NO: 60 - protein, 10 aa, Artificial
  1276 CDR1 Heavy Chain
GFTFNTFAMN

SEQ ID NO: 61 - protein, 17 aa, Artificial
  1276 CDR2 Heavy Chain
AITGSGGSTYYADSVKG

SEQ ID NO: 62 - protein, 13 aa, Artificial
  1276 CDR3 Heavy Chain
PITVVRGVSAFDI

SEQ ID NO: 63 - protein, 108 aa, Artificial
  1276 VL
EIVLTQSPGTLSLSPGERATLSCRASQSVSSSYLAWYQQKPGQAPRLLIYGASSRATGIPDRFSGSGSGTDFTLTISRLEPEDFAVYYCQQYGSSPITFGQGTRLEIK

SEQ ID NO: 64 - protein, 122 aa, Artificial
  1276 VH
EVQLLESGGGLVQPGGSLRLSCAASGFTFNTFAMNWVRQAPGKGLEWVSAITGSGGSTYYADSVKGRFTISRDNSKNTLYLQMNSLRAEDTAVYYCATPITVVRGVSAFDIWGQGTMVTVSS

SEQ ID NO: 65 - protein, 12 aa, Artificial
  849 CDR1 Light Chain
RASQSVSSSYLA

SEQ ID NO: 66 - protein, 7 aa, Artificial
  849 CDR2 Light Chain
GASSRAT

SEQ ID NO: 67 - protein, 9 aa, Artificial
  849 CDR3 Light Chain
QQYGSSPLT

SEQ ID NO: 68 - protein, 10 aa, Artificial
  849 CDR1 Heavy Chain
GFTFNTFAMN

SEQ ID NO: 69 - protein, 17 aa, Artificial
  849 CDR2 Heavy Chain
AISGSGGSTYYADSVKG

SEQ ID NO: 70 - protein, 11 aa, Artificial
  849 CDR3 Heavy Chain
LVRGVRDAFDI

SEQ ID NO: 71 - protein, 108 aa, Artificial
  849 VL
EIVLTQSPGTLSLSPGERATLSCRASQSVSSSYLAWYQQKPGQAPRLLIYGASSRATGIPDRFSGSGSGTDFTLTISRLEPEDFAVYYCQQYGSSPLTFGGGTKVEIK

SEQ ID NO: 72 - protein, 120 aa, Artificial
  849 VH
EVQLLESGGGLVQPGGSLRLSCAASGFTFNTFAMNWVRQAPGKGLEWVSAISGSGGSTYYADSVKGRFTISRDNSKNTLYLQMNSLRAEDTAVYYCAALVRGVRDAFDIWGQGTMVTVSS

SEQ ID NO: 73 - protein, 12 aa, Artificial
  531-02 CDR1 Light Chain
RASQSVSSSDLA

SEQ ID NO: 74 - protein, 7 aa, Artificial
  531-02 CDR2 Light Chain
GASSRAT

SEQ ID NO: 75 - protein, 9 aa, Artificial
  531-02 CDR3 Light Chain
QQYGSSPLT

SEQ ID NO: 76 - protein, 10 aa, Artificial
  531-02 CDR1 Heavy Chain
GFTFSRYVMS

SEQ ID NO: 77 - protein, 17 aa, Artificial
  531-02 CDR2 Heavy Chain
TISGSGGSTYYADSVKG

SEQ ID NO: 78 - protein, 8 aa, Artificial
  531-02 CDR3 Heavy Chain
GAFGAFDI

SEQ ID NO: 79 - protein, 108 aa, Artificial
  531-02 VL
EIVLTQSPGTLSLSPGERATLSCRASQSVSSSDLAWYQQKPGQAPRLLIYGASSRATGIPDRFSGSGSGTDFTLTISRLEPEDFAVYYCQQYGSSPLTFGGGTKVEIK

SEQ ID NO: 80 - protein, 117 aa, Artificial
  531-02 VH
EVQLLESGGGLVQPGGSLRLSCAASGFTFSRYVMSWVRQAPGKGLEWVSTISGSGGSTYYADSVKGRFTISRDNSKNTLFLQMNSLRAEDTAVYYCAEGAFGAFDIWGQGTMVTVSS

SEQ ID NO: 81 - protein, 12 aa, Artificial
  548-01 CDR1 Light Chain
RASQSVSSSYLV

SEQ ID NO: 82 - protein, 7 aa, Artificial
  548-01 CDR2 Light Chain
GASSRAT

SEQ ID NO: 83 - protein, 9 aa, Artificial
  548-01 CDR3 Light Chain
QQYGSSPIT

SEQ ID NO: 84 - protein, 10 aa, Artificial
  548-01 CDR1 Heavy Chain
KFTFNTYAMN

SEQ ID NO: 85 - protein, 17 aa, Artificial
  548-01 CDR2 Heavy Chain
AISGSGISSYYADSVNG

SEQ ID NO: 86 - protein, 13 aa, Artificial
  548-01 CDR3 Heavy Chain
PIVVVSIDMAFDI

SEQ ID NO: 87 - protein, 108 aa, Artificial
  548-01 VL
EIVLTQSPGTLSLSPGERATLSCRASQSVSSSYLVWYQQKPGQAPRLLIYGASSRATGIPDRFSGSGSGTDFTLTISRLEPEDFAVYYCQQYGSSPITFGQGTRLEIK

SEQ ID NO: 88 - protein, 122 aa, Artificial
  548-01 VH
EVQLLESGGGLVQPGGSLRLSCTASKFTFNTYAMNWVRQAPGKGLEWVSAISGSGISSYYADSVNGRFTISRDNSKNTLYLQMNSLRAEDTAVYYCATPIVVVSIDMAFDIWGQGTMVTVSS

SEQ ID NO: 89 - protein, 11 aa, Artificial
  548-02 CDR1 Light Chain
RASQSVSSYLA

SEQ ID NO: 90 - protein, 7 aa, Artificial
  548-02 CDR2 Light Chain
DASNRAT

SEQ ID NO: 91 - protein, 9 aa, Artificial
  548-02 CDR3 Light Chain
QQRSNWPLT

SEQ ID NO: 92 - protein, 10 aa, Artificial
  548-02 CDR1 Heavy Chain
KFTFNTYAMN

SEQ ID NO: 93 - protein, 17 aa, Artificial
  548-02 CDR2 Heavy Chain
AISGSGISSYYADSVNG

SEQ ID NO: 94 - protein, 13 aa, Artificial
  548-02 CDR3 Heavy Chain
PIVVVSIDMAFDI

SEQ ID NO: 95 - protein, 107 aa, Artificial
  548-02 VL
EIVLTQSPATLSLSPGERATLSCRASQSVSSYLAWYQQKPGQAPRLLIYDASNRATGIPARFSGSGSGTDFTLTISSLEPEDFAVYYCQQRSNWPLTFGGGTKVEIK

SEQ ID NO: 96 - protein, 122 aa, Artificial; identical to SEQ ID NO: 88
  548-02 VH

SEQ ID NO: 97 - protein, 12 aa, Artificial
  1289-02 CDR1 Light Chain
RASQSVSSSYLA

SEQ ID NO: 98 - protein, 7 aa, Artificial
  1289-02 CDR2 Light Chain
GASSRAT

SEQ ID NO: 99 - protein, 9 aa, Artificial
  1289-02 CDR3 Light Chain
QQYGSSPIT

SEQ ID NO: 100 - protein, 10 aa, Artificial
  1289-02 CDR1 Heavy Chain
GFTFSSFAMS

SEQ ID NO: 101 - protein, 17 aa, Artificial
  1289-02 CDR2 Heavy Chain
AISGSGGSTYYADSVKG

SEQ ID NO: 102 - protein, 13 aa, Artificial
  1289-02 CDR3 Heavy Chain
PITLVRGVGAFDI

SEQ ID NO: 103 - protein, 108 aa, Artificial; identical to SEQ ID NO: 63
  1289-02 VL

SEQ ID NO: 104 - protein, 122 aa, Artificial
  1289-02 VH
EVQLLESGGGLVQPGGSLRLSCAASGFTFSSFAMSWVRQAPGKGLEWVSAISGSGGSTYYADSVKGRFTISRDNSKNTLSLQMNSLRAEDTAVYYCATPITLVRGVGAFDIWGQGTMVTVSS

SEQ ID NO: 105 - protein, 12 aa, Artificial
  811-02 CDR1 Light Chain
RASQSVSSSYLA

SEQ ID NO: 106 - protein, 7 aa, Artificial
  811-02 CDR2 Light Chain
GASSRAT

SEQ ID NO: 107 - protein, 10 aa, Artificial
  811-02 CDR3 Light Chain
QQYGSSPPWT

SEQ ID NO: 108 - protein, 10 aa, Artificial
  811-02 CDR1 Heavy Chain
GFTFSTFAMN

SEQ ID NO: 109 - protein, 17 aa, Artificial
  811-02 CDR2 Heavy Chain
AISGSGGNTYYADSVKG

SEQ ID NO: 110 - protein, 12 aa, Artificial
  811-02 CDR3 Heavy Chain
IPVKLGDDAFDI

SEQ ID NO: 111 - protein, 109 aa, Artificial
  811-02 VL
EIVLTQSPGTLSLSPGERATLSCRASQSVSSSYLAWYQQKPGQAPRLLIYGASSRATGIPDRFSGSGSGTDFTLTISRLEPEDFAVYYCQQYGSSPPWTFGQGTKVEIK

SEQ ID NO: 112 - protein, 121 aa, Artificial
  811-02 VH
EVQLLESGGGLVQPGGSLRLSCAVSGFTFSTFAMNWVRQAPGKGLEWVSAISGSGGNTYYADSVKGRFIISRDNSKNTLYLQMNSLRAEDTAVYYCATIPVKLGDDAFDIWGQGTMVTVSS

SEQ ID NO: 113 - protein, 12 aa, Artificial
  566-01 CDR1 Light Chain
RASQSVSSSYLA

SEQ ID NO: 114 - protein, 7 aa, Artificial
  566-01 CDR2 Light Chain
GASSRAT

SEQ ID NO: 115 - protein, 9 aa, Artificial
  566-01 CDR3 Light Chain
QQYGSSPIT

SEQ ID NO: 116 - protein, 10 aa, Artificial
  566-01 CDR1 Heavy Chain
GFTFSTFAMS

SEQ ID NO: 117 - protein, 17 aa, Artificial
  566-01 CDR2 Heavy Chain
AISGSGGSTYYADSVRG

SEQ ID NO: 118 - protein, 12 aa, Artificial
  566-01 CDR3 Heavy Chain
PITMVRGEAFDI

SEQ ID NO: 119 - protein, 108 aa, Artificial; identical to SEQ ID NO: 63
  566-01 VL

SEQ ID NO: 120 - protein, 121 aa, Artificial
  566-01 VH
EVQLLESGGGLVQPGGSLRLSCVASGFTFSTFAMSWVRQAPGKGLEWVSAISGSGGSTYYADSVRGRFTVSRDNSKNTLYLQMNSLRAEDTAVYYCASPITMVRGEAFDIWGQGTMVTVSS

SEQ ID NO: 121 - protein, 12 aa, Artificial
  562 CDR1 Light Chain
RASQSVSSSYLA

SEQ ID NO: 122 - protein, 7 aa, Artificial
  562 CDR2 Light Chain
GASSRAT

SEQ ID NO: 123 - protein, 9 aa, Artificial
  562 CDR3 Light Chain
QQYGSSPIT

SEQ ID NO: 124 - protein, 10 aa, Artificial
  562 CDR1 Heavy Chain
GFTFSTFAMS

SEQ ID NO: 125 - protein, 17 aa, Artificial
  562 CDR2 Heavy Chain
AISGSGGSTYYADSVKG

SEQ ID NO: 126 - protein, 12 aa, Artificial
  562 CDR3 Heavy Chain
PITVVRGEAFDI

SEQ ID NO: 127 - protein, 108 aa, Artificial; identical to SEQ ID NO: 63
  562 VL

SEQ ID NO: 128 - protein, 121 aa, Artificial
  562 VH
EVQLLESGGGLVQPGGSLRLSCAASGFTFSTFAMSWVRQAPGKGLEWVSAISGSGGSTYYADSVKGRFTISRDNSENTLYLQMNSLRAEDTAVYYCASPITVVRGEAFDIWGQGTMVTVSS

SEQ ID NO: 129 - protein, 12 aa, Artificial
  193 CDR1 Light Chain
RASQSVSSSYIA

SEQ ID NO: 130 - protein, 7 aa, Artificial
  193 CDR2 Light Chain
GASSRAT

SEQ ID NO: 131 - protein, 9 aa, Artificial
  193 CDR3 Light Chain
QQYVNSPLT

SEQ ID NO: 132 - protein, 10 aa, Artificial
  193 CDR1 Heavy Chain
GFTFTSFAMS

SEQ ID NO: 133 - protein, 17 aa, Artificial
  193 CDR2 Heavy Chain
GISGSGGSTYYADSVKG

SEQ ID NO: 134 - protein, 11 aa, Artificial
  193 CDR3 Heavy Chain
LVRGVIIVFDI

SEQ ID NO: 135 - protein, 108 aa, Artificial
  193 VL
EIVLTQSPGTLSLSPGERATLSCRASQSVSSSYIAWYQQKPGQAPRLLIYGASSRATGIPDRFSGSGSGTDFSLTISRLEPEDFAVYYCQQYVNSPLTFGGGTKVEIK

SEQ ID NO: 136 - protein, 120 aa, Artificial
  193 VH
EVQLLESGGGLVLPGGSLRLSCAASGFTFTSFAMSWVRQAPGKGLEWVSGISGSGGSTYYADSVKGRFTISRDNSKNTLYLQMSSLRAEDTAVYYCASLVRGVIIVFDIWGQGTMVTVSS

SEQ ID NO: 137 - protein, 12 aa, Artificial
  88 CDR1 Light Chain
RASQSVSSSYLA

SEQ ID NO: 138 - protein, 7 aa, Artificial
  88 CDR2 Light Chain
GASSRAT

SEQ ID NO: 139 - protein, 9 aa, Artificial
  88 CDR3 Light Chain
QQYGSSPLT

SEQ ID NO: 140 - protein, 10 aa, Artificial
  88 CDR1 Heavy Chain
GFTFSTFAMS

SEQ ID NO: 141 - protein, 17 aa, Artificial
  88 CDR2 Heavy Chain
AISGSGGGTYYADSVKG

SEQ ID NO: 142 - protein, 12 aa, Artificial
  88 CDR3 Heavy Chain
YIVATIADAFDI

SEQ ID NO: 143 - protein, 108 aa, Artificial; identical to SEQ ID NO: 71
  88 VL

SEQ ID NO: 144 - protein, 121 aa, Artificial
  88 VH
EVQLLESGGGLVQPGGSLRLSCAASGFTFSTFAMSWVRQAPGKGLEWVSAISGSGGGTYYADSVKGRFTISRDNSKNTLYLQMNSLRAEDTAVYYCATYIVATIADAFDIWGQGTMVTVSS

SEQ ID NO: 145 - protein, 12 aa, Artificial
  045 CDR1 Light Chain
RASQSVSSSYLA

SEQ ID NO: 146 - protein, 7 aa, Artificial
  045 CDR2 Light Chain
GASSRAT

SEQ ID NO: 147 - protein, 9 aa, Artificial
  045 CDR3 Light Chain
QHYGSSPLT

SEQ ID NO: 148 - protein, 10 aa, Artificial
  045 CDR1 Heavy Chain
GFTFNSYAMS

SEQ ID NO: 149 - protein, 17 aa, Artificial
  045 CDR2 Heavy Chain
AISGSGGITYYADSVKG

SEQ ID NO: 150 - protein, 11 aa, Artificial
  045 CDR3 Heavy Chain
MVRGVIVNFDY

SEQ ID NO: 151 - protein, 108 aa, Artificial
  045 VL
EIVLTQSPGTLSLSPGERATLSCRASQSVSSSYLAWYQQKPGQAPRLLIYGASSRATGIPDRFSGSGSGTDFTLTISRLEPEDFAVYYCQHYGSSPLTFGGGTKVEIK

SEQ ID NO: 152 - protein, 120 aa, Artificial
  045 VH
EVQLLESGGGLVQPGGSLRLSCAASGFTFNSYAMSWVRQAPGKGLEWVSAISGSGGITYYADSVKGRFTISRDNSKNTLYLQMSSLRAEDTAVYYCASMVRGVIVNFDYWGQGTLVTVSS

SEQ ID NO: 153 - protein, 12 aa, Artificial
  044 CDR1 Light Chain
RASQSVSSSYLA

SEQ ID NO: 154 - protein, 7 aa, Artificial
  044 CDR2 Light Chain
GASSRAT

SEQ ID NO: 155 - protein, 9 aa, Artificial
  044 CDR3 Light Chain
QQYGSSPLT

SEQ ID NO: 156 - protein, 10 aa, Artificial
  044 CDR1 Heavy Chain
GFTFSSYAMS

SEQ ID NO: 157 - protein, 17 aa, Artificial
  044 CDR2 Heavy Chain
AISGSGGNTYYADSVKG

SEQ ID NO: 158 - protein, 11 aa, Artificial
  044 CDR3 Heavy Chain
MVRGVFINFDY

SEQ ID NO: 159 - protein, 108 aa, Artificial; identical to SEQ ID NO: 71
  044 VL

SEQ ID NO: 160 - protein, 120 aa, Artificial
  044 VH
EVQLLESGGGLVQPGGSLRLSCAASGFTFSSYAMSWVRQAPGKGLEWVSAISGSGGNTYYADSVKGRSTISRDNSKNTLYLQMNSLRAEDTAVYYCASMVRGVFINFDYWGQGTLVTVSS

SEQ ID NO: 161 - protein, 12 aa, Artificial
  002 CDR1 Light Chain
RASQSVSSSYLA

SEQ ID NO: 162 - protein, 7 aa, Artificial
  002 CDR2 Light Chain
GASSRAT

SEQ ID NO: 163 - protein, 8 aa, Artificial
  002 CDR3 Light Chain
QQYGSSLT

SEQ ID NO: 164 - protein, 10 aa, Artificial
  002 CDR1 Heavy Chain
GFTFSSYAMS

SEQ ID NO: 165 - protein, 17 aa, Artificial
  002 CDR2 Heavy Chain
AISGSGGSTYYADSVKG

SEQ ID NO: 166 - protein, 11 aa, Artificial
  002 CDR3 Heavy Chain
MVRGVIINFDY

SEQ ID NO: 167 - protein, 107 aa, Artificial
  002 VL
EIVLTQSPGTLSLSPGERATLSCRASQSVSSSYLAWYQQKPGQAPRLLIYGASSRATGIPDRFSGSGSGTDFTLTISRLEPEDFAVYYCQQYGSSLTFGQGTRLEIK

SEQ ID NO: 168 - protein, 120 aa, Artificial
  002 VH
EVQLLESGGGLVQPGGSLRLSCAASGFTFSSYAMSWVRQAPGKGLEWVSAISGSGGSTYYADSVKGRFTISRDNSKNTLYLQMNSLRAEDTAVYYCAVMVRGVIINFDYWGQGTLVTVSS

SEQ ID NO: 169 - protein, 831 aa, Artificial
  full human Sortilin sequence isoform 1
MERPWGAADGLSRWPHGLGLLLLLQLLPPSTLSQDRLDAPPPPAAPLPRWSGPIGVSWGLRAAAAGGAFPRGGRWRRSAPGEDEECGRVRDFVAKLANNTHQHVFDDLRGSVSLSWVGDSTGVILVLTTFHVPLVIMTFGQSKLYRSEDYGKNFKDITDLINNTFIRTEFGMAIGPENSGKVVLTAEVSGGSRGGRIFRSSDFAKNFVQTDLPFHPLTQMMYSPQNSDYLLALSTENGLWVSKNFGGKWEEIHKAVCLAKWGSDNTIFFTTYANGSCKADLGALELWRTSDLGKSFKTIGVKIYSFGLGGRFLFASVMADKDTTRRIHVSTDQGDTWSMAQLPSVGQEQFYSILAANDDMVFMHVDEPGDTGFGTIFTSDDRGIVYSKSLDRHLYTTTGGETDFTNVTSLRGVYITSVLSEDNSIQTMITFDQGGRWTHLRKPENSECDATAKNKNECSLHIHASYSISQKLNVPMAPLSEPNAVGIVIAHGSVGDAISVMVPDVYISDDGGYSWTKMLEGPHYYTILDSGGIIVAIEHSSRPINVIKFSTDEGQCWQTYTFTRDPIYFTGLASEPGARSMNISIWGFTESFLTSQWVSYTIDFKDILERNCEEKDYTIWLAHSTDPEDYEDGCILGYKEQFLRLRKSSVCQNGRDYVVTKQPSICLCSLEDFLCDFGYYRPENDSKCVEQPELKGHDLEFCLYGREEHLTTNGYRKIPGDKCQGGVNPVREVKDLKKKCTSNFLSPEKQNSKSNSVPIILAIVGLMLVTVVAGVLIVKKYVCGGRFLVHRYSVLQQHAEANGVDGVDALDTASHTNKSGYHDDSDEDLLE

SEQ ID NO: 170 - protein, 88 aa, Artificial
  D region as identified by  present invention
HYYTILDSGGIIVAIEHSSRPINVIKFSTDEGQCWQTYTFTRDPIYFTGLASEPGARSMNISIWGFTESFLTSQWVSYTIDFKDILER

SEQ ID NO: 171 - protein, 700 aa, Artificial
  Sortilin hSORTECDBAP
SAPGEDEECGRVRDFVAKLANNTHQHVFDDLRGSVSLSWVGDSTGVILVLTTFHVPLVIMTFGQSKLYRSEDYGKNFKDITDLINNTFIRTEFGMAIGPENSGKVVLTAEVSGGSRGGRIFRSSDFAKNFVQTDLPFHPLTQMMYSPQNSDYLLALSTENGLWVSKNFGGKWEEIHKAVCLAKWGSDNTIFFTTYANGSCKADLGALELWRTSDLGKSFKTIGVKIYSFGLGGRFLFASVMADKDTTRRIHVSTDQGDTWSMAQLPSVGQEQFYSILAANDDMVFMHVDEPGDTGFGTIFTSDDRGIVYSKSLDRHLYTTTGGETDFTNVTSLRGVYITSVLSEDNSIQTMITFDQGGRWTHLRKPENSECDATAKNKNECSLHIHASYSISQKLNVPMAPLSEPNAVGIVIAHGSVGDAISVMVPDVYISDDGGYSWTKMLEGPHYYTILDSGGIIVAIEHSSRPINVIKFSTDEGQCWQTYTFTRDPIYFTGLASEPGARSMNISIWGFTESFLTSQWVSYTIDFKDILERNCEEKDYTIWLAHSTDPEDYEDGCILGYKEQFLRLRKSSVCQNGRDYVVTKQPSICLCSLEDFLCDFGYYRPENDSKCVEQPELKGHDLEFCLYGREEHLTTNGYRKIPGDKCQGGVNPVREVKDLKKKCTSNFLSPEKQNSKSNGSAGGSGGLNDIFEAQKIEWHE

SEQ ID NO: 172 - protein, 700 aa, Artificial
  Sortilin SORTECDBAP_hBACK
SAPGEDEECGRVRDFVAKLANNTHQHIFNDLSGSVSLSWVGDSTGVILVLTTFQVPIFMITIGQSKLYRSEDYGKNFKDITDLINNTFIRSDFGIAIGPENSGKVVLTADVSGSHGSRIFRSSDFAKNFVQQELPFVPLMQIMYSPQNSDYLLALSNKNELWVSKNFGGKWEKLYDTVCLAKWGSDNTIFFTANHNGSCSNDRGMLELWRTSDLGKSFKTIGSKIYSFGLGGRFLFASVMTGKGTLRAIHVSTDQGDTWSMAQLPPVGHEQFYSILAANDDMVFMHVDEPGDSGFGTIFTSDDRGIVYSKSLERHLYTTTGGETDFTNVTSLRGVYITSILAEDKSVQSMITFDQGGRWTHLRKPENSKCDATARDPEKCSLHIHAAYSIATGLNVPMLPLSEPNAVGIVIAHGSVGDAISVMRPDVYISDDGGYSWTKALEGPHHYTILDSGGIIVAVEQNAHQGVNQIKFSTDEGQCWQTYNFTKDPIFFTGLASEPGARSMNISIWGYRSSLFHQYWISYTIDFKDILERNCEEKDYTIWLAHSTDPEDYEDGCILGYKEQFLRLRKSSVCQNGRDYVVTKQPSICLCSLEDFLCDFGYYRPENDSKCVEQPELKGHDLEFCLYGREEHLTTNGYRKIPGDKCQGGVNPVREVKDLKKKCTSNFLSPEKQNSKSNGSAGGSGGLNDIFEAQKIEWHE

SEQ ID NO: 173 - protein, 700 aa, Artificial
  Sortilin  SORTECDBAP_tetra
RSTEQGESCSGLLGADAKLAGNTHQHIFNDLSGSVSLAWVGDGTGVILALTTFQVPIFMITIGQSKLYRSEDYGKSFEDVTNLINNTFIRSDFGIAIGPENSGKVILTADVSGSHGSRIFVSSDFGKSFTHQELPFVPLMQITYNPENSNVLLALSNKNELWLSEDFGTNWKKLYDTVCLAKWGRKGTIFFTANHNGSCSNDRGMLELERTTDYGKSFKTVASKIYSFGLGGKFLFASVMTGKGTLRAIHVSVDDGDTWNMAQLPPVGHEQFYSILAANDEMVFMHVDEPGDSGFGTIYVSDDRGTVYSKSLERHLYTTTGGETDFINVTSLRGVFTTSILAEDKSVQSVISFDQGGEWVPLRKPADSKCDATARDPEKCSLHIHAAYSIATGLNVPMLPLSEPNAVGLVLAHGSVGDAISVMRPDVYVSDDGGYTWIKALEGPHHYAILDSGGLLVAVEQNAHQGVNQIKFSTDEGQCWGVYNFTKDPIFFTGLASEPGARSMNVSLWGYRSSLFHQYWISFTIDFRDLITRNCTDKDYVQWLAHSDDISDPNDGCMLGYKEKFLRLKKDSVCLNGRDYEVNTQPTPCLCTLDDFLCDFGYYRKENSSECVEQPDLKGKVLEFCLHGTEEELLTNGYRKIPGDKCEGGQIPERKEINLRRRCVSDLLGPEFLVKKSSGSAGGSGGLNDIFEAQKIEWHE

SEQ ID NO: 174 - protein, 701 aa, Artificial
  Sortilin  SORTECDBAP_hB01-05
SAPGEDEECGRVRDFVAKLANNTHQHVFDDLRGSVSLSWVGDSTGVILVLTTFHVPLVIMTFGQSKLYRSEDYGKNFKDITDLINNTFIRTEFGMAIGPENSGKVVLTAEVSGGSRGGRIFRSSDFAKNFVQTDLPFHPLTQMMYSPQNSDYLLALSTENGLWVSKNFGGKWEEIHKAVCLAKWGSDNTIFFTTYANGSCKADLGALELWRTSDLGKSFKTIGVKIYSFGLGGRFLFASVMADKDTTRRIHVSTDQGDTWSMAQLPPVGHEQFYSILAANDEMVFMHVDEPGDSGFGTIYVSDDRGTVYSKSLERHLYTTTGGETDFINVTSLRGVFTTSILAEDKSVQSVISFDQGGEWVPLRKPADSKCDATARDPEKCSLHIHAAYSIATGLNVPMLPLSEPNAVGLVLAHGSVGDAISVMRPDVYVSDDGGYTWIKALEGPHHYAILDSGGLLVAVEQNAHQGVNQIKFSTDEGQCWGVYNFTKDPIFFTGLASEPGARSMNVSLWGYRSSLFHQYWISFTIDFRDLITRNCTDKDYVQWLAHSDDISDPNDGCMLGYKEKFLRLKKDSVCLNGRDYEVNTQPTPCLCTLDDFLCDFGYYRKENSSECVEQPDLKGKVLEFCLHGTEEELLTNGYRKIPGDKCEGGQIPERKEINLRRRCVSDLLGPEFLVKKSSGSAGGSGGLNDIFEAQKIEWHE

SEQ ID NO: 175 - protein, 700 aa, Artificial
  Sortilin  SORTECDBAP_hRIM
SAPGEDEECGRVRDFVAKLANNTHQHVFDDLRGSVSLAWVGDGTGVILALTTFQVPIFMITIGQSKLYRSEDYGKNFKDITDLINNTFIRSDFGIAIGPENSGKVILTADVSGSHGSRIFRSSDFAKNFVQTDLPFVPLMQITYNPENSNVLLALSNKNELWVSKNFGGKWEEIHDTVCLAKWGRKGTIFFTANHNGSCSNDRGMLELWRTSDLGKSFKTIGVKIYSFGLGGKFLFASVMTGKGTLRRIHVSTDQGDTWSMAQLPSVGHEQFYSILAANDEMVFMHVDEPGDSGFGTIFTSDDRGIVYSKSLDRHLYTTTGGETDFINVTSLRGVFTTSILAEDKSIQTMITFDQGGRWTHLRKPENSECDATAKNKNECSLHIHAAYSIATGLNVPMLPLSEPNAVGLVLAHGSVGDAISVMRPDVYISDDGGYSWTKMLEGPHHYAILDSGGLLVAVEQNAHQGVNVIKFSTDEGQCWQTYTFTRDPIFFTGLASEPGARSMNVSLWGYRSSLFHQQWVSYTIDFKDILERNCEEKDYTIWLAHSTDPEDYEDGCILGYKEQFLRLRKSSVCQNGRDYVVTKQPSICLCSLEDFLCDFGYYRPENDSKCVEQPELKGHDLEFCLYGREEHLTTNGYRKIPGDKCQGGVNPVREVKDLKKKCTSNFLSPEKQNSKSNGSAGGSGGLNDIFEAQKIEWHE

SEQ ID NO: 176 - protein, 699 aa, Artificial
  Sortilin  SORTECDBAP_hB06-10
RSTEQGESCSGLLGADAKLAGNTHQHIFNDLSGSVSLAWVGDGTGVILALTTFQVPIFMITIGQSKLYRSEDYGKSFEDVTNLINNTFIRSDFGIAIGPENSGKVILTADVSGSHGSRIFVSSDFGKSFTHQELPFVPLMQITYNPENSNVLLALSNKNELWLSEDFGTNWKKLYDTVCLAKWGRKGTIFFTANHNGSCSNDRGMLELERTTDYGKSFKTVASKIYSFGLGGKFLFASVMTGKGTLRAIHVSVDDGDTWNMAQLPSVGQEQFYSILAANDDMVFMHVDEPGDTGFGTIFTSDDRGIVYSKSLDRHLYTTTGGETDFTNVTSLRGVYITSVLSEDNSIQTMITFDQGGRWTHLRKPENSECDATAKNKNECSLHIHASYSISQKLNVPMAPLSEPNAVGIVIAHGSVGDAISVMVPDVYISDDGGYSWTKMLEGPHYYTILDSGGIIVAIEHSSRPINVIKFSTDEGQCWQTYTFTRDPIYFTGLASEPGARSMNISIWGFTESFLTSQWVSYTIDFKDILERNCEEKDYTIWLAHSTDPEDYEDGCILGYKEQFLRLRKSSVCQNGRDYVVTKQPSICLCSLEDFLCDFGYYRPENDSKCVEQPELKGHDLEFCLYGREEHLTTNGYRKIPGDKCQGGVNPVREVKDLKKKCTSNFLSPEKQNSKSNGSAGGSGGLNDIFEAQKIEWHE

SEQ ID NO: 177 - protein, 700 aa, Artificial
  Sortilin  SORTECDBAP_hB12390
SAPGEDEECGRVRDFVAKLANNTHQHVFDDLRGSVSLSWVGDSTGVILVLTTFHVPLVIMTFGQSKLYRSEDYGKNFKDITDLINNTFIRTEFGMAIGPENSGKVVLTAEVSGGSRGGRIFRSSDFAKNFVQTDLPFHPLTQMMYSPQNSDYLLALSTENGLWVSKNFGGKWEEIHKTVCLAKWGRKGTIFFTANHNGSCSNDRGMLELERTTDYGKSFKTVASKIYSFGLGGKFLFASVMTGKGTLRAIHVSVDDGDTWNMAQLPPVGHEQFYSILAANDEMVFMHVDEPGDSGFGTIYVSDDRGTVYSKSLERHLYTTTGGETDFINVTSLRGVFTTSILAEDKSVQSVISFDQGGEWVPLRKPADSKCDATARDPEKCSLHIHAAYSIATGLNVPMLPLSEPNAVGLVLAHGSVGDAISVMRPDVYVSDDGGYTWIKALEGPHYYTILDSGGIIVAIEHSSRPINVIKFSTDEGQCWQTYTFTRDPIYFTGLASEPGARSMNISIWGFTESFLTSQWVSYTIDFKDILERNCEEKDYTIWLAHSTDPEDYEDGCILGYKEQFLRLRKSSVCQNGRDYVVTKQPSICLCSLEDFLCDFGYYRPENDSKCVEQPELKGHDLEFCLYGREEHLTTNGYRKIPGDKCQGGVNPVREVKDLKKKCTSNFLSPEKQNSKSNGSAGGSGGLNDIFEAQKIEWHE

SEQ ID NO: 178 - protein, 700 aa, Artificial
  Sortilin  SORTECDBAP_hB45678
RSTEQGESCSGLLGADAKLAGNTHQHIFNDLSGSVSLAWVGDGTGVILALTTFQVPIFMITIGQSKLYRSEDYGKSFEDVTNLINNTFIRSDFGIAIGPENSGKVILTADVSGSHGSRIFVSSDFGKSFTHQELPFVPLMQITYNPENSNVLLALSNKNELWLSEDFGTNWKKLYDAVCLAKWGSDNTIFFTTYANGSCKADLGALELWRTSDLGKSFKTIGVKIYSFGLGGRFLFASVMADKDTTRRIHVSTDQGDTWSMAQLPSVGQEQFYSILAANDDMVFMHVDEPGDTGFGTIFTSDDRGIVYSKSLDRHLYTTTGGETDFTNVTSLRGVYITSVLSEDNSIQTMITFDQGGRWTHLRKPENSECDATAKNKNECSLHIHASYSISQKLNVPMAPLSEPNAVGIVIAHGSVGDAISVMVPDVYISDDGGYSWTKMLEGPHHYAILDSGGLLVAVEQNAHQGVNQIKFSTDEGQCWGVYNFTKDPIFFTGLASEPGARSMNVSLWGYRSSLFHQYWISFTIDFRDLITRNCEEKDYTIWLAHSTDPEDYEDGCILGYKEQFLRLRKSSVCQNGRDYVVTKQPSICLCSLEDFLCDFGYYRPENDSKCVEQPELKGHDLEFCLYGREEHLTTNGYRKIPGDKCQGGVNPVREVKDLKKKCTSNFLSPEKQNSKSNGSAGGSGGLNDIFEAQKIEWHE

SEQ ID NO: 179 - protein, 763 aa, Artificial
  Sortilin  SORTECD_HIS
MERPWGAADGLSRWPHGLGLLLLLQLLPPSTLSQDRLDAPPPPAAPLPRWSGPIGVSWGLRAAAAGGAFPRGGRWRRSAPGEDEECGRVRDFVAKLANNTHQHVFDDLRGSVSLSWVGDSTGVILVLTTFHVPLVIMTFGQSKLYRSEDYGKNFKDITDLINNTFIRTEFGMAIGPENSGKVVLTAEVSGGSRGGRIFRSSDFAKNFVQTDLPFHPLTQMMYSPQNSDYLLALSTENGLWVSKNFGGKWEEIHKAVCLAKWGSDNTIFFTTYANGSCKADLGALELWRTSDLGKSFKTIGVKIYSFGLGGRFLFASVMADKDTTRRIHVSTDQGDTWSMAQLPSVGQEQFYSILAANDDMVFMHVDEPGDTGFGTIFTSDDRGIVYSKSLDRHLYTTTGGETDFTNVTSLRGVYITSVLSEDNSIQTMITFDQGGRWTHLRKPENSECDATAKNKNECSLHIHASYSISQKLNVPMAPLSEPNAVGIVIAHGSVGDAISVMVPDVYISDDGGYSWTKMLEGPHYYTILDSGGIIVAIEHSSRPINVIKFSTDEGQCWQTYTFTRDPIYFTGLASEPGARSMNISIWGFTESFLTSQWVSYTIDFKDILERNCEEKDYTIWLAHSTDPEDYEDGCILGYKEQFLRLRKSSVCQNGRDYVVTKQPSICLCSLEDFLCDFGYYRPENDSKCVEQPELKGHDLEFCLYGREEHLTTNGYRKIPGDKCQGGVNPVREVKDLKKKCTSNFLSPEKQNSKSNHHHHHHHH

SEQ ID NO: 180 - protein, 177 aa, Artificial
  A region
SAPGEDEECGRVRDFVAKLANNTHQHVFDDLRGSVSLSWVGDSTGVILVLTTFHVPLVIMTFGQSKLYRSEDYGKNFKDITDLINNTFIRTEFGMAIGPENSGKVVLTAEVSGGSRGGRIFRSSDFAKNFVQTDLPFHPLTQMMYSPQNSDYLLALSTENGLWVSKNFGGKWEEIHK

SEQ ID NO: 181 - protein, 6 aa, Artificial
  A region amino acids 109-114
RGSVSL

SEQ ID NO: 182 - protein, 28 aa, Artificial
  A region amino acides 126-153
VLTTFHVPLVIMTFGQSKLYRSEDYGKN

SEQ ID NO: 183 - protein, 19 aa, Artificial
  A region amino acides 126-144
VLTTFHVPLVIMTFGQSKL

SEQ ID NO: 184 - protein, 6 aa, Artificial
  A region amino acides 154-159
FKDITD

SEQ ID NO: 185 - protein, 3 aa, Artificial
  D region amino acids 570-572
TGL

SEQ ID NO: 186 - protein, 10 aa, Artificial
  D region amino acids 588-597
FTESFLTSQW

SEQ ID NO: 187 - protein, 5 aa, Artificial
  D region amino acids 593-597
LTSQW

SEQ ID NO: 188 - protein, 696 aa, Artificial
  Sequences used for HDX experiments
SAPGEDEECGRVRDFVAKLANNTHQHVFDDLRGSVSLSWVGDSTGVILVLTTFHVPLVIMTFGQSKLYRSEDYGKNFKDITDLINNTFIRTEFGMAIGPENSGKVVLTAEVSGGSRGGRIFRSSDFAKNFVQTDLPFHPLTQMMYSPQNSDYLLALSTENGLWVSKNFGGKWEEIHKAVCLAKWGSDNTIFFTTYANGSCKADLGALELWRTSDLGKSFKTIGVKIYSFGLGGRFLFASVMADKDTTRRIHVSTDQGDTWSMAQLPSVGQEQFYSILAANDDMVFMHVDEPGDTGFGTIFTSDDRGIVYSKSLDRHLYTTTGGETDFTNVTSLRGVYITSVLSEDNSIQTMITFDQGGRWTHLRKPENSECDATAKNKNECSLHIHASYSISQKLNVPMAPLSEPNAVGIVIAHGSVGDAISVMVPDVYISDDGGYSWTKMLEGPHYYTILDSGGIIVAIEHSSRPINVIKFSTDEGQCWQTYTFTRDPIYFTGLASEPGARSMNISIWGFTESFLTSQWVSYTIDFKDILERNCEEKDYTIWLAHSTDPEDYEDGCILGYKEQFLRLRKSSVCQNGRDYVVTKQPSICLCSLEDFLCDFGYYRPENDSKCVEQPELKGHDLEFCLYGREEHLTTNGYRKIPGDKCQGGVNPVREVKDLKKKCTSNFLSPEKQNSKSNSGSAMIEGRGVGHHHHHH